European Patent Application EP 4 431 619 A2, published September 18, 2024. Title: Method of identifying feature of test body and microRNA cancer marker. Applicant: Kabushiki Kaisha Toshiba. The sequence listing filed with the application follows.

SEQUENCE LISTING (40 sequences)

SEQ ID NO: 1 - DNA, 23 bp, synthetic construct
  misc_feature 1..23: note = 17_hsa-miR-199a-5p_C-T
  source 1..23: mol_type = other DNA
cccagtgttcagactatctgttc

SEQ ID NO: 2 - DNA, 19 bp, synthetic construct
  misc_feature 1..19: note = 9_hsa-miR-1260b_A-G
  source 1..19: mol_type = other DNA
atcccaccgctgccaccat

SEQ ID NO: 3 - DNA, 23 bp, synthetic construct
  misc_feature 1..23: note = 18_hsa-miR-146b-5p_A-G
  source 1..23: mol_type = other DNA
tgagaactgaattccatgggctg

SEQ ID NO: 4 - DNA, 20 bp, synthetic construct
  misc_feature 1..20: note = 9_hsa-miR-33b-5p_C-T
  source 1..20: mol_type = other DNA
gtgcattgttgttgcattgc

SEQ ID NO: 5 - DNA, 22 bp, synthetic construct
  misc_feature 1..22: note = 20_hsa-miR-15b-5p_A-G
  source 1..22: mol_type = other DNA
tagcagcacatcatggtttgca

SEQ ID NO: 6 - DNA, 22 bp, synthetic construct
  misc_feature 1..22: note = 10_hsa-miR-92b-3p_C-T
  source 1..22: mol_type = other DNA
tattgcacttgtcccggcctcc

SEQ ID NO: 7 - DNA, 23 bp, synthetic construct
  misc_feature 1..23: note = 12_hsa-miR-106a-5p_C-T,
  source 1..23: mol_type = other DNA
aaaagtgcttatagtgcaggtag

SEQ ID NO: 8 - DNA, 22 bp, synthetic construct
  misc_feature 1..22: note = 11_hsa-miR-98-5p_A-G,
  source 1..22: mol_type = other DNA
tgaggtagtaggttgtattgtt

SEQ ID NO: 9 - DNA, 22 bp, synthetic construct
  misc_feature 1..22: note = 13_hsa-miR-130a-3p_A-G,
  source 1..22: mol_type = other DNA
cagtgcaatgttgaaagggcat

SEQ ID NO: 10 - DNA, 22 bp, synthetic construct
  misc_feature 1..22: note = 11_hsa-miR-26a-5p_C-T,
  source 1..22: mol_type = other DNA
ttcaagtaattcaggataggct

SEQ ID NO: 11 - DNA, 22 bp, synthetic construct
  misc_feature 1..22: note = 16_hsa-let-7d-5p_C-T,
  source 1..22: mol_type = other DNA
agaggtagtaggttgtatagtt

SEQ ID NO: 12 - DNA, 22 bp, synthetic construct
  misc_feature 1..22: note = 17_hsa-let-7g-5p_A-G,
  source 1..22: mol_type = other DNA
tgaggtagtagtttgtgcagtt

SEQ ID NO: 13 - DNA, 22 bp, synthetic construct
  misc_feature 1..22: note = 9_hsa-miR-501-3p_C-T,
  source 1..22: mol_type = other DNA
aatgcacctgggcaaggattct

SEQ ID NO: 14 - DNA, 22 bp, synthetic construct
  misc_feature 1..22: note = 7_hsa-miR-335-3p_A-G,
  source 1..22: mol_type = other DNA
tttttcgttattgctcctgacc

SEQ ID NO: 15 - DNA, 18 bp, synthetic construct
  misc_feature 1..18: note = 16_hsa-miR-320e_A-G,
  source 1..18: mol_type = other DNA
aaagctgggttgagaggg

SEQ ID NO: 16 - DNA, 18 bp, synthetic construct
  misc_feature 1..18: note = 6_hsa-miR-1827_C-T,
  source 1..18: mol_type = other DNA
tgaggtagtagattgaat

SEQ ID NO: 17 - DNA, 22 bp, synthetic construct
  misc_feature 1..22: note = 10_hsa-miR-1273h-3p_C-T,
  source 1..22: mol_type = other DNA
ctgcagacttgacctcccaggc

SEQ ID NO: 18 - DNA, 22 bp, synthetic construct
  misc_feature 1..22: note = 10_hsa-miR-200a-3p_C-T,
  source 1..22: mol_type = other DNA
taacactgtttggtaacgatgt

SEQ ID NO: 19 - DNA, 22 bp, synthetic construct
  misc_feature 1..22: note = 1_hsa-miR-99a-5p_A-G,
  source 1..22: mol_type = other DNA
gacccgtagatccgatcttgtg

SEQ ID NO: 20 - DNA, 22 bp, synthetic construct
  misc_feature 1..22: note = 17_hsa-miR-4510_A-G,
  source 1..22: mol_type = other DNA
tgagggagtaggatgtgtggtt

SEQ ID NO: 21 - RNA, 23 nt, unidentified
  misc_feature 1..23: note = 17_hsa-miR-199a-5p_C-U
  source 1..23: mol_type = other RNA; note = human
cccagtgttcagactatctgttc

SEQ ID NO: 22 - RNA, 19 nt, unidentified
  misc_feature 1..19: note = 9_hsa-miR-1260b_A-G
  source 1..19: mol_type = other RNA; note = Human
atcccaccgctgccaccat

SEQ ID NO: 23 - RNA, 23 nt, unidentified
  misc_feature 1..23: note = 18_hsa-miR-146b-5p_A-G,
  source 1..23: mol_type = other RNA; note = Human
tgagaactgaattccatgggctg

SEQ ID NO: 24 - RNA, 20 nt, unidentified
  misc_feature 1..20: note = 9_hsa-miR-33b-5p_C-U,
  source 1..20: mol_type = other RNA; note = Human
gtgcattgttgttgcattgc

SEQ ID NO: 25 - RNA, 22 nt, unidentified
  misc_feature 1..22: note = 20_hsa-miR-15b-5p_A-G,
  source 1..22: mol_type = other RNA; note = Human
tagcagcacatcatggtttgca

SEQ ID NO: 26 - RNA, 22 nt, unidentified
  misc_feature 1..22: note = 10_hsa-miR-92b-3p_C-U,
  source 1..22: mol_type = other RNA; note = Human
tattgcacttgtcccggcctcc

SEQ ID NO: 27 - RNA, 23 nt, unidentified
  misc_feature 1..23: note = 12_hsa-miR-106a-5p_C-U,
  source 1..23: mol_type = other RNA; note = Human
aaaagtgcttatagtgcaggtag

SEQ ID NO: 28 - RNA, 22 nt, unidentified
  misc_feature 1..22: note = 11_hsa-miR-98-5p_A-G,
  source 1..22: mol_type = other RNA; note = Human
tgaggtagtaggttgtattgtt

SEQ ID NO: 29 - RNA, 22 nt, unidentified
  misc_feature 1..22: note = 13_hsa-miR-130a-3p_A-G,
  source 1..22: mol_type = other RNA; note = Human
cagtgcaatgttgaaagggcat

SEQ ID NO: 30 - RNA, 22 nt, unidentified
  misc_feature 1..22: note = 11_hsa-miR-26a-5p_C-U,
  source 1..22: mol_type = other RNA; note = Human
ttcaagtaattcaggataggct

SEQ ID NO: 31 - RNA, 22 nt, unidentified
  misc_feature 1..22: note = 16_hsa-let-7d-5p_C-U,
  source 1..22: mol_type = other RNA; note = Human
agaggtagtaggttgtatagtt

SEQ ID NO: 32 - RNA, 22 nt, unidentified
  misc_feature 1..22: note = 17_hsa-let-7g-5p_A-G,
  source 1..22: mol_type = other RNA; note = Human
tgaggtagtagtttgtgcagtt

SEQ ID NO: 33 - RNA, 22 nt, unidentified
  misc_feature 1..22: note = 9_hsa-miR-501-3p_C-U,
  source 1..22: mol_type = other RNA; note = Human
aatgcacctgggcaaggattct

SEQ ID NO: 34 - RNA, 22 nt, unidentified
  misc_feature 1..22: note = 7_hsa-miR-335-3p_A-G,
  source 1..22: mol_type = other RNA; note = Human
tttttcgttattgctcctgacc

SEQ ID NO: 35 - RNA, 18 nt, unidentified
  misc_feature 1..18: note = 16_hsa-miR-320e_A-G,
  source 1..18: mol_type = other RNA; note = Human
aaagctgggttgagaggg

SEQ ID NO: 36 - RNA, 18 nt, unidentified
  misc_feature 1..18: note = 6_hsa-miR-1827_C-U,
  source 1..18: mol_type = other RNA; note = Human
tgaggtagtagattgaat

SEQ ID NO: 37 - RNA, 22 nt, unidentified
  misc_feature 1..22: note = 10_hsa-miR-1273h-3p_C-U,
  source 1..22: mol_type = other RNA; note = Human
ctgcagacttgacctcccaggc

SEQ ID NO: 38 - RNA, 22 nt, unidentified
  misc_feature 1..22: note = 10_hsa-miR-200a-3p_C-U,
  source 1..22: mol_type = other RNA; note = Human
taacactgtttggtaacgatgt

SEQ ID NO: 39 - RNA, 22 nt, unidentified
  misc_feature 1..22: note = 1_hsa-miR-99a-5p_A-G,
  source 1..22: mol_type = other RNA; note = Human
gacccgtagatccgatcttgtg

SEQ ID NO: 40 - RNA, 22 nt, unidentified
  misc_feature 1..22: note = 17_hsa-miR-4510_A-G,
  source 1..22: mol_type = other RNA; note = Human
tgagggagtaggatgtgtggtt